European Patent Specification EP 3 964 529 B1, published March 26, 2025. Title: IMMUNOLOGICAL REAGENTS. Applicant: MABQUEST SA. Application PCT/IB2017/000031. The sequence listing filed with the application follows.

SEQUENCE LISTING (292 sequences)

SEQ ID NO: 1 - protein, 5 aa, Artificial Sequence
  Synthetic
DDFLH

SEQ ID NO: 2 - protein, 5 aa, Artificial Sequence
  Synthetic
NYYIH

SEQ ID NO: 3 - protein, 5 aa, Artificial Sequence
  Synthetic
NYYIH

SEQ ID NO: 4 - protein, 5 aa, Artificial Sequence
  Synthetic
SNWMH

SEQ ID NO: 5 - protein, 5 aa, Artificial Sequence
  Synthetic
RYWMH

SEQ ID NO: 6 - protein, 5 aa, Artificial Sequence
  Synthetic
SNWMH

SEQ ID NO: 7 - protein, 5 aa, Artificial Sequence
  Synthetic
NSYIH

SEQ ID NO: 8 - protein, 5 aa, Artificial Sequence
  Synthetic
NYWIG

SEQ ID NO: 9 - protein, 5 aa, Artificial Sequence
  Synthetic
SYAMS

SEQ ID NO: 10 - protein, 6 aa, Artificial Sequence
  Synthetic
SDYAWN

SEQ ID NO: 11 - protein, 5 aa, Artificial Sequence
  Synthetic
SYWIN

SEQ ID NO: 12 - protein, 5 aa, Artificial Sequence
  Synthetic
SSYIH

SEQ ID NO: 13 - protein, 5 aa, Artificial Sequence
  Synthetic
NHGMS

SEQ ID NO: 14 - protein, 5 aa, Artificial Sequence
  Synthetic
NYWIG

SEQ ID NO: 15 - protein, 5 aa, Artificial Sequence
  Synthetic
DSYIH

SEQ ID NO: 16 - protein, 5 aa, Artificial Sequence
  Synthetic
DTYIH

SEQ ID NO: 17 - protein, 5 aa, Artificial Sequence
  Synthetic
NFYIH

SEQ ID NO: 18 - protein, 5 aa, Artificial Sequence
  Synthetic
DSYIH

SEQ ID NO: 19 - protein, 5 aa, Artificial Sequence
  Synthetic
DDFLH

SEQ ID NO: 20 - protein, 5 aa, Artificial Sequence
  Synthetic
SYFMS

SEQ ID NO: 21 - protein, 5 aa, Artificial Sequence
  Synthetic
NHGMS

SEQ ID NO: 22 - protein, 5 aa, Artificial Sequence
  Synthetic
NYWIG

SEQ ID NO: 23 - protein, 5 aa, Artificial Sequence
  Synthetic
SFAMS

SEQ ID NO: 24 - protein, 17 aa, Artificial Sequence
  Synthetic
RIDPANGESRYAPKFQD

SEQ ID NO: 25 - protein, 17 aa, Artificial Sequence
  Synthetic
SIYPNYGDTNYNQKVKD

SEQ ID NO: 26 - protein, 17 aa, Artificial Sequence
  Synthetic
SIYPNYGETNYNQEFKG

SEQ ID NO: 27 - protein, 17 aa, Artificial Sequence
  Synthetic
AVNPGNSDTTYNQKFKG

SEQ ID NO: 28 - protein, 17 aa, Artificial Sequence
  Synthetic
NIDPSDSTTHYNPKFRD

SEQ ID NO: 29 - protein, 17 aa, Artificial Sequence
  Synthetic
AVYPGNSDTTYNQNFKG

SEQ ID NO: 30 - protein, 17 aa, Artificial Sequence
  Synthetic
WISPGDGSTNYNEKFKG

SEQ ID NO: 31 - protein, 17 aa, Artificial Sequence
  Synthetic
DIYPGGGYTNYNEKFKG

SEQ ID NO: 32 - protein, 17 aa, Artificial Sequence
  Synthetic
TISGGGADTYYLDNVKG

SEQ ID NO: 33 - protein, 16 aa, Artificial Sequence
  Synthetic
YINYSGYTNYNPFLKS

SEQ ID NO: 34 - protein, 17 aa, Artificial Sequence
  Synthetic
NIYPGSSSTDYNEKFKS

SEQ ID NO: 35 - protein, 17 aa, Artificial Sequence
  Synthetic
WIFPGDGKTNYNEKFRD

SEQ ID NO: 36 - protein, 17 aa, Artificial Sequence
  Synthetic
SINTGGYSTYYPDNVKG

SEQ ID NO: 37 - protein, 17 aa, Artificial Sequence
  Synthetic
DIYPGSEYENYNEKFKG

SEQ ID NO: 38 - protein, 17 aa, Artificial Sequence
  Synthetic
RIDPAHGNVIYASKFRD

SEQ ID NO: 39 - protein, 17 aa, Artificial Sequence
  Synthetic
RIDLANDDILYASKFQG

SEQ ID NO: 40 - protein, 17 aa, Artificial Sequence
  Synthetic
SIYPNYGDTAYNQKFKD

SEQ ID NO: 41 - protein, 17 aa, Artificial Sequence
  Synthetic
RIDPARDNIIYASKFRD

SEQ ID NO: 42 - protein, 17 aa, Artificial Sequence
  Synthetic
RIDPANGESRYAPQFQD

SEQ ID NO: 43 - protein, 17 aa, Artificial Sequence
  Synthetic
GISTGGADTYYADSMKG

SEQ ID NO: 44 - protein, 17 aa, Artificial Sequence
  Synthetic
SISGGGDNTYYPDNLKG

SEQ ID NO: 45 - protein, 17 aa, Artificial Sequence
  Synthetic
DIYPGGDHKNYNEKFKD

SEQ ID NO: 46 - protein, 17 aa, Artificial Sequence
  Synthetic
TITGGGVNTYYPDTVKG

SEQ ID NO: 47 - protein, 12 aa, Artificial Sequence
  Synthetic
TDYRGYYYAMDY

SEQ ID NO: 48 - protein, 8 aa, Artificial Sequence
  Synthetic
GYSYAMDY

SEQ ID NO: 49 - protein, 8 aa, Artificial Sequence
  Synthetic
GYSYAMDY

SEQ ID NO: 50 - protein, 10 aa, Artificial Sequence
  Synthetic
GRSYDGSFDY

SEQ ID NO: 51 - protein, 15 aa, Artificial Sequence
  Synthetic
DLDDFYVGSHEDFDY

SEQ ID NO: 52 - protein, 10 aa, Artificial Sequence
  Synthetic
GRSYDGSFDY

SEQ ID NO: 53 - protein, 8 aa, Artificial Sequence
  Synthetic
EEYDYDNY

SEQ ID NO: 54 - protein, 8 aa, Artificial Sequence
  Synthetic
GYDFVLDR

SEQ ID NO: 55 - protein, 9 aa, Artificial Sequence
  Synthetic
QRGENLFAH

SEQ ID NO: 56 - protein, 11 aa, Artificial Sequence
  Synthetic
YGGSYPWNFDV

SEQ ID NO: 57 - protein, 8 aa, Artificial Sequence
  Synthetic
GLYWYFDV

SEQ ID NO: 58 - protein, 8 aa, Artificial Sequence
  Synthetic
NDFDRGVY

SEQ ID NO: 59 - protein, 8 aa, Artificial Sequence
  Synthetic
DDYNWFAY

SEQ ID NO: 60 - protein, 8 aa, Artificial Sequence
  Synthetic
GYDFVLDH

SEQ ID NO: 61 - protein, 10 aa, Artificial Sequence
  Synthetic
IYYDYGEGDF

SEQ ID NO: 62 - protein, 10 aa, Artificial Sequence
  Synthetic
IYYDYGEGDY

SEQ ID NO: 63 - protein, 8 aa, Artificial Sequence
  Synthetic
GYSYAMDY

SEQ ID NO: 64 - protein, 10 aa, Artificial Sequence
  Synthetic
IYYDYGEGDY

SEQ ID NO: 65 - protein, 12 aa, Artificial Sequence
  Synthetic
TDYRGYYYAMDY

SEQ ID NO: 66 - protein, 12 aa, Artificial Sequence
  Synthetic
LSHYYDGIPLDC

SEQ ID NO: 67 - protein, 13 aa, Artificial Sequence
  Synthetic
VRQLGLHRAAMDY

SEQ ID NO: 68 - protein, 8 aa, Artificial Sequence
  Synthetic
GFDFVLDY

SEQ ID NO: 69 - protein, 12 aa, Artificial Sequence
  Synthetic
QAIYDGHYVLDY

SEQ ID NO: 70 - protein, 17 aa, Artificial Sequence
  Synthetic
KSSQSVLYSSNQKNYLA

SEQ ID NO: 71 - protein, 11 aa, Artificial Sequence
  Synthetic
SASQGISDGLN

SEQ ID NO: 72 - protein, 11 aa, Artificial Sequence
  Synthetic
SASQGISNGLN

SEQ ID NO: 73 - protein, 11 aa, Artificial Sequence
  Synthetic
KASQDINKYIA

SEQ ID NO: 74 - protein, 16 aa, Artificial Sequence
  Synthetic
RSSQSIVYSNGNTYLE

SEQ ID NO: 75 - protein, 11 aa, Artificial Sequence
  Synthetic
KASQDINKYMA

SEQ ID NO: 76 - protein, 11 aa, Artificial Sequence
  Synthetic
KASQNVGTNVG

SEQ ID NO: 77 - protein, 17 aa, Artificial Sequence
  Synthetic
KSSQSLFNSETQKNYLA

SEQ ID NO: 78 - protein, 11 aa, Artificial Sequence
  Synthetic
LASQTIGTWLA

SEQ ID NO: 79 - protein, 16 aa, Artificial Sequence
  Synthetic
RSSQTIVHNNGDTYLE

SEQ ID NO: 80 - protein, 17 aa, Artificial Sequence
  Synthetic
KSSQSLFNSGTRKNYLA

SEQ ID NO: 81 - protein, 11 aa, Artificial Sequence
  Synthetic
KASQNVDTNVA

SEQ ID NO: 82 - protein, 17 aa, Artificial Sequence
  Synthetic
KSSQSLLNSGNQKNYLT

SEQ ID NO: 83 - protein, 17 aa, Artificial Sequence
  Synthetic
KSSQSLFNSGTRKSYLA

SEQ ID NO: 84 - protein, 11 aa, Artificial Sequence
  Synthetic
HASQNINVWLS

SEQ ID NO: 85 - protein, 11 aa, Artificial Sequence
  Synthetic
HASQNINVWLS

SEQ ID NO: 86 - protein, 11 aa, Artificial Sequence
  Synthetic
SASQGISGDLN

SEQ ID NO: 87 - protein, 11 aa, Artificial Sequence
  Synthetic
HASQNINVWLS

SEQ ID NO: 88 - protein, 17 aa, Artificial Sequence
  Synthetic
KSSQSVLYSSNQKNYLA

SEQ ID NO: 89 - protein, 15 aa, Artificial Sequence
  Synthetic
RASESVDNSGVSFLT

SEQ ID NO: 90 - protein, 11 aa, Artificial Sequence
  Synthetic
KASQSVSDDVS

SEQ ID NO: 91 - protein, 17 aa, Artificial Sequence
  Synthetic
KSSQSLFNSGTRKNYLA

SEQ ID NO: 92 - protein, 11 aa, Artificial Sequence
  Synthetic
RTSGNIHNYLA

SEQ ID NO: 93 - protein, 7 aa, Artificial Sequence
  Synthetic
WASTRES

SEQ ID NO: 94 - protein, 7 aa, Artificial Sequence
  Synthetic
HTSTLHS

SEQ ID NO: 95 - protein, 7 aa, Artificial Sequence
  Synthetic
HTSTLHS

SEQ ID NO: 96 - protein, 7 aa, Artificial Sequence
  Synthetic
YTSTLRP

SEQ ID NO: 97 - protein, 7 aa, Artificial Sequence
  Synthetic
KVSHRFS

SEQ ID NO: 98 - protein, 7 aa, Artificial Sequence
  Synthetic
YTSTLRP

SEQ ID NO: 99 - protein, 7 aa, Artificial Sequence
  Synthetic
SASYRYN

SEQ ID NO: 100 - protein, 7 aa, Artificial Sequence
  Synthetic
WASTRES

SEQ ID NO: 101 - protein, 7 aa, Artificial Sequence
  Synthetic
AATSLAD

SEQ ID NO: 102 - protein, 7 aa, Artificial Sequence
  Synthetic
KISNRFF

SEQ ID NO: 103 - protein, 7 aa, Artificial Sequence
  Synthetic
WASTRDS

SEQ ID NO: 104 - protein, 7 aa, Artificial Sequence
  Synthetic
SASYRYN

SEQ ID NO: 105 - protein, 7 aa, Artificial Sequence
  Synthetic
WASTRES

SEQ ID NO: 106 - protein, 7 aa, Artificial Sequence
  Synthetic
WASTRET

SEQ ID NO: 107 - protein, 7 aa, Artificial Sequence
  Synthetic
KASNLHT

SEQ ID NO: 108 - protein, 7 aa, Artificial Sequence
  Synthetic
KASNLHT

SEQ ID NO: 109 - protein, 7 aa, Artificial Sequence
  Synthetic
HTSSLHS

SEQ ID NO: 110 - protein, 7 aa, Artificial Sequence
  Synthetic
KASNLHT

SEQ ID NO: 111 - protein, 7 aa, Artificial Sequence
  Synthetic
WASTRES

SEQ ID NO: 112 - protein, 7 aa, Artificial Sequence
  Synthetic
AASNQGS

SEQ ID NO: 113 - protein, 7 aa, Artificial Sequence
  Synthetic
SAFFRYP

SEQ ID NO: 114 - protein, 7 aa, Artificial Sequence
  Synthetic
WASTRES

SEQ ID NO: 115 - protein, 7 aa, Artificial Sequence
  Synthetic
NVKTLTD

SEQ ID NO: 116 - protein, 8 aa, Artificial Sequence
  Synthetic
HQYLSSYT

SEQ ID NO: 117 - protein, 9 aa, Artificial Sequence
  Synthetic
QQYSKFPLT

SEQ ID NO: 118 - protein, 9 aa, Artificial Sequence
  Synthetic
QQYSKFPLT

SEQ ID NO: 119 - protein, 8 aa, Artificial Sequence
  Synthetic
LQYDNLWT

SEQ ID NO: 120 - protein, 9 aa, Artificial Sequence
  Synthetic
FQGSHVPYT

SEQ ID NO: 121 - protein, 8 aa, Artificial Sequence
  Synthetic
LQYDNLWT

SEQ ID NO: 122 - protein, 9 aa, Artificial Sequence
  Synthetic
QQYNTYPWT

SEQ ID NO: 123 - protein, 8 aa, Artificial Sequence
  Synthetic
KQSYTLRT

SEQ ID NO: 124 - protein, 9 aa, Artificial Sequence
  Synthetic
QQLYSTPWT

SEQ ID NO: 125 - protein, 9 aa, Artificial Sequence
  Synthetic
FQGSHVPYT

SEQ ID NO: 126 - protein, 8 aa, Artificial Sequence
  Synthetic
KQSYNLYT

SEQ ID NO: 127 - protein, 9 aa, Artificial Sequence
  Synthetic
QQYNNYPYT

SEQ ID NO: 128 - protein, 9 aa, Artificial Sequence
  Synthetic
QSDYSYPLT

SEQ ID NO: 129 - protein, 8 aa, Artificial Sequence
  Synthetic
MQSYNLRT

SEQ ID NO: 130 - protein, 9 aa, Artificial Sequence
  Synthetic
QQGQSWPLT

SEQ ID NO: 131 - protein, 9 aa, Artificial Sequence
  Synthetic
QQGQSYPLT

SEQ ID NO: 132 - protein, 9 aa, Artificial Sequence
  Synthetic
QYYSKDLLT

SEQ ID NO: 133 - protein, 9 aa, Artificial Sequence
  Synthetic
QQGQSWPLT

SEQ ID NO: 134 - protein, 8 aa, Artificial Sequence
  Synthetic
HQYLSSYT

SEQ ID NO: 135 - protein, 9 aa, Artificial Sequence
  Synthetic
QQTKEVPWT

SEQ ID NO: 136 - protein, 9 aa, Artificial Sequence
  Synthetic
QQDYSSPLT

SEQ ID NO: 137 - protein, 8 aa, Artificial Sequence
  Synthetic
MQSFNLRT

SEQ ID NO: 138 - protein, 9 aa, Artificial Sequence
  Synthetic
QQFWSIPWT

SEQ ID NO: 139 - protein, 117 aa, Artificial Sequence
  Synthetic
QMQLVQSGPEVKKPGTSVKVSCKASGFTFTNYWIGWVRQAPGQALEWMGDIYPGGGYTNYNEKFKGRVTITADKSTSTAYMELSSLRSEDTAVYYCARGYDFVLDRWGQGTTVTVSS

SEQ ID NO: 140 - protein, 117 aa, Artificial Sequence; identical to SEQ ID NO: 139
  Synthetic

SEQ ID NO: 141 - protein, 117 aa, Artificial Sequence; identical to SEQ ID NO: 139
  Synthetic

SEQ ID NO: 142 - protein, 117 aa, Artificial Sequence; identical to SEQ ID NO: 139
  Synthetic

SEQ ID NO: 143 - protein, 117 aa, Artificial Sequence
  Synthetic
QVQLVQSGAEVKKPGASVKVSCKASGYTFTNYWIGWVRQAPGQGLEWMGDIYPGGGYTNYNEKFKGRVTITADKSTSTAYMELSSLRSEDTAVYYCARGYDFVLDRWGQGTTVTVSS

SEQ ID NO: 144 - protein, 117 aa, Artificial Sequence
  Synthetic
EVQLVQSGAEVKKHGESLKISCKGSGYSFTNYWIGWVRQATGQGLEWMGDIYPGGGYTNYNEKFKGRVTITADKSTSTAYMELSSLRSEDTAVYYCARGYDFVLDRWGQGTTVTVSS

SEQ ID NO: 145 - protein, 117 aa, Artificial Sequence
  Synthetic
QMQLVQSGAEVKKTGSSVKVSCKASGYTFTNYWIGWVRQMPGKGLEWMGDIYPGGGYTNYNEKFKGRVTITADKSTSTAYMELSSLRSEDTAVYYCARGYDFVLDRWGQGTTVTVSS

SEQ ID NO: 146 - protein, 117 aa, Artificial Sequence
  Synthetic
QVQLVQSGSELKKPGASVKVSCKASGYTFTNYWIGWVRQAPGKGLEWMGDIYPGGGYTNYNEKFKGRVTITADKSTSTAYMELSSLRSEDTAVYYCARGYDFVLDRWGQGTTVTVSS

SEQ ID NO: 147 - protein, 117 aa, Artificial Sequence
  Synthetic
QVQLVQSGAEVKKPGASVKVSCKASGYTFTNYWIGWVRQAPGQGLEWMGDIYPGGGYTNYNEKFKGRVTMTRDTSTSTVYMELSSLRSEDTAVYYCARGYDFVLDRWGQGTLVTVSS

SEQ ID NO: 148 - protein, 117 aa, Artificial Sequence
  Synthetic
QVQLVQSGAEVKKPGASVKVSCKAAGYTFTNYWIGWVRQAPGQGLEWMGDIYPGGGYTNYNEKFKGRVTMTADTSTSTVYMELSSLRSEDTAVYYCARGYDFVLDRWGQGTLVTVSS

SEQ ID NO: 149 - protein, 117 aa, Artificial Sequence
  Synthetic
QVQLVQSGAEVKKPGASVKVSCKASGYTFTNYWIGWVRQAPGQGLEWIGDIYPGGGYTNYNEKFKGRVTMTADTSTSTVYMELSSLRSEDTAVYYCARGYDFVLDRWGQGTLVTVSS

SEQ ID NO: 150 - protein, 117 aa, Artificial Sequence
  Synthetic
QVQLVQSGAEVKKPGASVKVSCKASGYTFTNYWIGWIRQAPGQGLEWIGDIYPGGGYTNYNEKFKGRATLTADTSTSTVYMEVSSLRSEDTAVYYCARGYDFVLDRWGQGTLVTVSS

SEQ ID NO: 151 - protein, 112 aa, Artificial Sequence
  Synthetic
DVVMTQSPAFLSVTPGEKVTITCKSSQSLFNSETQKNYLAWYQQKPGQPPKLLIYWASTRESGVPSRFSGSGSGTDFTLTISSLQPEDFATYYCKQSYTLRTFGGGTKLEIK

SEQ ID NO: 152 - protein, 112 aa, Artificial Sequence; identical to SEQ ID NO: 151
  Synthetic

SEQ ID NO: 153 - protein, 112 aa, Artificial Sequence
  Synthetic
DVVMTQSPAFLSVTPGEKVTITCKSSQSLFNSETQKNYLAWYQQKPGQPPKLLIYWASTRESGVPSRFSGSGSGTDFTFTISSLEAEDAATYYCKQSYTLRTFGGGTKLEIK

SEQ ID NO: 154 - protein, 112 aa, Artificial Sequence
  Synthetic
DVVMTQSPAFLSVTPGEKVTITCKSSQSLFNSETQKNYLAWYQQKPGQAPRLLIYWASTRESGVPSRFSGSGSGTDFTFTISSLEAEDAATYYCKQSYTLRTFGGGTKLEIK

SEQ ID NO: 155 - protein, 112 aa, Artificial Sequence
  Synthetic
DVVMTQSPAFLSVTPGEKVTITCKSSQSLFNSETQKNYLAWYQQKPGQAPRLLIYWASTRESGVPSRFSGSGSGTDFTLTISSLQPEDFATYYCKQSYTLRTFGGGTKLEIK

SEQ ID NO: 156 - protein, 112 aa, Artificial Sequence
  Synthetic
DIQMTQSPSSLSASVGDRVTITCKSSQSLFNSETQKNYLAWYQQKPGQPPKLLIYWASTRESGVPSRFSGSGSGTDFTLTISSLQPEDFATYYCKQSYTLRTFGGGTKLEIK

SEQ ID NO: 157 - protein, 112 aa, Artificial Sequence; identical to SEQ ID NO: 151
  Synthetic

SEQ ID NO: 158 - protein, 112 aa, Artificial Sequence; identical to SEQ ID NO: 153
  Synthetic

SEQ ID NO: 159 - protein, 112 aa, Artificial Sequence
  Synthetic
DIVMTQSPDSLAVSLGERATINCKSSQSLFNSETQKNYLAWYQQKPGQPPKLLIYWASTRESGVPDRFSGSGSGTDFTLTISSLQAEDVAVYYCKQSYTLRTFGQGTKLEIK

SEQ ID NO: 160 - protein, 112 aa, Artificial Sequence
  Synthetic
DIVMTQSPDSLAVSLGERATITCKSSQSLFNSETQKNYLAWYQQKPGQPPKLLIFWASTRESGVPDRFLGSGSGTDFTLTISSLQAEDVAVYYCKQSYTLRTFGQGTKLEIK

SEQ ID NO: 161 - protein, 112 aa, Artificial Sequence; identical to SEQ ID NO: 159
  Synthetic

SEQ ID NO: 162 - protein, 112 aa, Artificial Sequence
  Synthetic
DIVMTQSPDSLAVSLGERATITCKSSQSLFNSETQKNYLAWYQQKPGQPPKLLIFWASTRESGVPDRFSGSGSGTDFTLTISSLQAEDVAVYYCKQSYTLRTFGQGTKLEIK

SEQ ID NO: 163 - protein, 112 aa, Artificial Sequence
  Synthetic
DIVMTQSPDSLAVSLGERATMTCKSSQSLFNSETQKNYLAWYQQKPGQPPKLLIFWASTRESGVPDRFSGSGSGTDFTLTISSVQAEDVAVYYCKQSYTLRTFGQGTKLEIK

SEQ ID NO: 164 - protein, 117 aa, Artificial Sequence
  Synthetic
EVQLVQSGAEVKKPGESLKISCKGSGYSFTNFYIHWVRQAPGQRLEWMGSIYPNYGDTAYNQKFKDRFVFSLDTSVSTAYLQISSLKAEDTAVYYCARGYSYAMDYWGQGTTVTVSS

SEQ ID NO: 165 - protein, 117 aa, Artificial Sequence
  Synthetic
EVQLVQSGAEVKKPGESLKISCKGSGYSFTNFYIHWVRQARGQRLEWIGSIYPNYGDTAYNQKFKDRFVFSLDTSVSTAYLQISSLKAEDTAVYYCARGYSYAMDYWGQGTTVTVSS

SEQ ID NO: 166 - protein, 117 aa, Artificial Sequence; identical to SEQ ID NO: 164
  Synthetic

SEQ ID NO: 167 - protein, 117 aa, Artificial Sequence
  Synthetic
EVQLVQSGAEVKKPGATVKISCKVSGYTFTNFYIHWVRQARGQRLEWIGSIYPNYGDTAYNQKFKDRVTITADKSTSTAYMELSSLRSEDTAVYYCARGYSYAMDYWGQGTTVTVSS

SEQ ID NO: 168 - protein, 117 aa, Artificial Sequence
  Synthetic
EVQLVQSGAEVKKPGATVKISCKVSGYTFTNFYIHWVRQAPGKGLEWMGSIYPNYGDTAYNQKFKDRVTITADKSTSTAYMELSSLRSEDTAVYYCARGYSYAMDYWGQGTTVTVSS

SEQ ID NO: 169 - protein, 117 aa, Artificial Sequence
  Synthetic
EVQLVQSGAEVKKPGESLKISCKGSGYSFTNFYIHWVRQMPGKGLEWMGSIYPNYGDTAYNQKFKDRVTITADKSTSTAYMELSSLRSEDTAVYYCARGYSYAMDYWGQGTTVTVSS

SEQ ID NO: 170 - protein, 117 aa, Artificial Sequence
  Synthetic
EVQLVQSGAEVKKPGESLKISCKGSGYSFTNFYIHWVRQMPGKGLEWMGSIYPNYGDTAYNQKFKDRFVFSLDTSVSTAYLQISSLKAEDTAVYYCARGYSYAMDYWGQGTTVTVSS

SEQ ID NO: 171 - protein, 117 aa, Artificial Sequence; identical to SEQ ID NO: 170
  Synthetic

SEQ ID NO: 172 - protein, 117 aa, Artificial Sequence
  Synthetic
QVQLVQSGAEVKKPGASVKVSCKASGYTFTNFYIHWVRQAPGQGLEWMGSIYPNYGDTAYNQKFKDRVTMTRDTSTSTVYMELSSLRSEDTAVYYCARGYSYAMDYWGQGTLVTVSS

SEQ ID NO: 173 - protein, 117 aa, Artificial Sequence
  Synthetic
QVQLVQSGAEVKKPGASVKVSCKASGYTFTNFYIHWVRQAPGQGLEWMGSIYPNYGDTAYNQKFKDRVTMTVDKSTSTVYMELRSLRSEDTAVYYCARGYSYAMDYWGQGTLVTVSS

SEQ ID NO: 174 - protein, 117 aa, Artificial Sequence
  Synthetic
QVQLVQSGAEVKKPGASVKVSCKASGYTFTNFYIHWVKQAHGQGLEWMGSIYPNYGDTAYNQKFKDRVTMTVDKSTSTVYMELRSLRSEDTAVYYCARGYSYAMDYWGQGTLVTVSS

SEQ ID NO: 175 - protein, 117 aa, Artificial Sequence
  Synthetic
QVQLVQSGAEVKKPGASVKVSCKASGYTFTNFYIHWVRQAPGQGLEWIGSIYPNYGDTAYNQKFKDRVTMTVDTSTSTVYMELSSLRSEDTAVYYCARGYSYAMDYWGQGTLVTVSS

SEQ ID NO: 176 - protein, 117 aa, Artificial Sequence
  Synthetic
QVQLVQSGAEVKKPGASVKMSCKASGYTFTNFYIHWVRQAPGQGLEWIGSIYPNYGDTAYNQKFKDRATLTVDTSTSTAYMELSSLRSEDTAVYYCARGYSYAMDYWGQGTLVTVSS

SEQ ID NO: 177 - protein, 117 aa, Artificial Sequence
  Synthetic
QVQLVQSGAEVKKPGASVKMSCKASGYTFTNFYIHWVRQAPGQGLEWIGSIYPNYGDTAYNQKFKDRATLTVDKSTSTAYMELSSLRSEDTAVYYCARGYSYAMDYWGQGTLVTVSS

SEQ ID NO: 178 - protein, 107 aa, Artificial Sequence
  Synthetic
DIQMTQSPSSVSASVGDRVTITCSASQGISGDLNWYQQKPGQAPRLLIYHTSSLHSGVPSRFSGSGSGTDFTLTISSLQPEDFATYYCQYYSKDLLTFGGGTKLEIK

SEQ ID NO: 179 - protein, 107 aa, Artificial Sequence
  Synthetic
DIQMTQSPSSLSASVGDRVTITCSASQGISGDLNWYQQKPGKTPKLLIYHTSSLHSGVPSRFSGSGSGTDFTLTISSLQPEDFATYYCQYYSKDLLTFGGGTKLEIK

SEQ ID NO: 180 - protein, 107 aa, Artificial Sequence
  Synthetic
DIQMTQSPSSVSASVGDRVTITCSASQGISGDLNWYQQKPGKAPKLLIYHTSSLHSGVPSRFSGSGSGTDFTLTISSLQPEDFATYYCQYYSKDLLTFGGGTKLEIK

SEQ ID NO: 181 - protein, 107 aa, Artificial Sequence
  Synthetic
DIQMTQSPSSVSASVGDRVTITCSASQGISGDLNWYQQKPGQAPRLLIYHTSSLHSGVPSRFSGSGSGTEFTLTISRLEPEDFAVYYCQYYSKDLLTFGGGTKLEIK

SEQ ID NO: 182 - protein, 107 aa, Artificial Sequence
  Synthetic
DIQMTQSPSTLSASVGDRVTITCSASQGISGDLNWYQQKPGQAPRLLIYHTSSLHSGVPSRFSGSGSGTDFTLTISSLQPEDFATYYCQYYSKDLLTFGGGTKLEIK

SEQ ID NO: 183 - protein, 107 aa, Artificial Sequence
  Synthetic
DIQMTQSPSSVSASVGDRVTITCSASQGISGDLNWYQQKPGQAPRLLIYHTSSLHSGIPARFSGSGSGTDFTLTISRLEPEDFAVYYCQYYSKDLLTFGGGTKLEIK

SEQ ID NO: 184 - protein, 107 aa, Artificial Sequence
  Synthetic
DIQMTQSPSTLSASVGDRVTITCSASQGISGDLNWYQQKPGKTPKLLIYHTSSLHSGVPSRFSGSGSGTDFTLTISSLQPEDFATYYCQYYSKDLLTFGGGTKLEIK

SEQ ID NO: 185 - protein, 107 aa, Artificial Sequence
  Synthetic
DIQMTQSPSTLSASVGDRVTITCSASQGISGDLNWYQQKPGQAPRLLIYHTSSLHSGIPARFSGSGSGTDFTLTISSLQPEDFAVYYCQYYSKDLLTFGGGTKLEIK

SEQ ID NO: 186 - protein, 107 aa, Artificial Sequence
  Synthetic
DIQMTQSPSSLSASVGDRVTITCSASQGISGDLNWYQQKPGKAPKLLIYHTSSLHSGVPSRFSGSGSGTDFTLTISSLQPEDFATYYCQYYSKDLLTFGGGTKLEIK

SEQ ID NO: 187 - protein, 107 aa, Artificial Sequence
  Synthetic
DIQMTQSPSSLSASVGDRVTITCSASQGISGDLNWYQQKPGKAVKLLIYHTSSLHSGVPLRFSGSGSGTDYTLTISSLQPEDFATYYCQYYSKDLLTFGGGTKLEIK

SEQ ID NO: 188 - protein, 107 aa, Artificial Sequence
  Synthetic
DIQMTQSPSSLSASVGDRVTITCSASQGISGDLNWYQQKSDGAVKLLIYHTSSLHSGVPLRFSGSGSGTDYTLTISSLQPEDFATYYCQYYSKDLLTFGGGTKLEIK

SEQ ID NO: 189 - protein, 107 aa, Artificial Sequence
  Synthetic
DIQMTQSPSSLSASVGDRVTITCSASQGISGDLNWYQQKPGKAPKLLIYHTSSLHSGVPSRFSGSGSGTDYTLTISSLQPEDFATYYCQYYSKDLLTFGGGTKLEIK

SEQ ID NO: 190 - protein, 107 aa, Artificial Sequence
  Synthetic
DIQMTQSPSSLSASVGDRVTITCSASQGISGDLNWYQQKPGKAVKLLIYHTSSLHSGVPSRFSGSGSGTDYTLTISSLQPEDFATYYCQYYSKDLLTFGGGTKLELK

SEQ ID NO: 191 - DNA, 15 bp, Artificial Sequence
  Synthetic
gatgattttttacat

SEQ ID NO: 192 - DNA, 351 bp, Artificial Sequence
  Synthetic
cagatgcagctggtgcagagcggcccggaagtgaaaaaaccgggcaccagcgtgaaagtgagctgcaaagcgagcggctttacctttaccaactattggattggctgggtgcgccaggcgccgggccaggcgctggaatggatgggcgatatttatccgggcggcggctataccaactataacgaaaaatttaaaggccgcgtgaccattaccgcggataaaagcaccagcaccgcgtatatggaactgagcagcctgcgcagcgaagataccgcggtgtattattgcgcgcgcggctatgattttgtgctggatcgctggggccagggcaccaccgtgaccgtgagcagc

SEQ ID NO: 193 - DNA, 351 bp, Artificial Sequence; identical to SEQ ID NO: 192
  Synthetic

SEQ ID NO: 194 - DNA, 351 bp, Artificial Sequence; identical to SEQ ID NO: 192
  Synthetic

SEQ ID NO: 195 - DNA, 351 bp, Artificial Sequence; identical to SEQ ID NO: 192
  Synthetic

SEQ ID NO: 196 - DNA, 351 bp, Artificial Sequence
  Synthetic
caggtgcagctggtgcagagcggcgcggaagtgaaaaaaccgggcgcgagcgtgaaagtgagctgcaaagcgagcggctatacctttaccaactattggattggctgggtgcgccaggcgccgggccagggcctggaatggatgggcgatatttatccgggcggcggctataccaactataacgaaaaatttaaaggccgcgtgaccattaccgcggataaaagcaccagcaccgcgtatatggaactgagcagcctgcgcagcgaagataccgcggtgtattattgcgcgcgcggctatgattttgtgctggatcgctggggccagggcaccaccgtgaccgtgagcagc

SEQ ID NO: 197 - DNA, 351 bp, Artificial Sequence
  Synthetic
gaagtgcagctggtgcagagcggcgcggaagtgaaaaaacatggcgaaagcctgaaaattagctgcaaaggcagcggctatagctttaccaactattggattggctgggtgcgccaggcgaccggccagggcctggaatggatgggcgatatttatccgggcggcggctataccaactataacgaaaaatttaaaggccgcgtgaccattaccgcggataaaagcaccagcaccgcgtatatggaactgagcagcctgcgcagcgaagataccgcggtgtattattgcgcgcgcggctatgattttgtgctggatcgctggggccagggcaccaccgtgaccgtgagcagc

SEQ ID NO: 198 - DNA, 351 bp, Artificial Sequence
  Synthetic
cagatgcagctggtgcagagcggcgcggaagtgaaaaaaaccggcagcagcgtgaaagtgagctgcaaagcgagcggctatacctttaccaactattggattggctgggtgcgccagatgccgggcaaaggcctggaatggatgggcgatatttatccgggcggcggctataccaactataacgaaaaatttaaaggccgcgtgaccattaccgcggataaaagcaccagcaccgcgtatatggaactgagcagcctgcgcagcgaagataccgcggtgtattattgcgcgcgcggctatgattttgtgctggatcgctggggccagggcaccaccgtgaccgtgagcagc

SEQ ID NO: 199 - DNA, 351 bp, Artificial Sequence
  Synthetic
caggtgcagctggtgcagagcggcagcgaactgaaaaaaccgggcgcgagcgtgaaagtgagctgcaaagcgagcggctatacctttaccaactattggattggctgggtgcgccaggcgccgggcaaaggcctggaatggatgggcgatatttatccgggcggcggctataccaactataacgaaaaatttaaaggccgcgtgaccattaccgcggataaaagcaccagcaccgcgtatatggaactgagcagcctgcgcagcgaagataccgcggtgtattattgcgcgcgcggctatgattttgtgctggatcgctggggccagggcaccaccgtgaccgtgagcagc

SEQ ID NO: 200 - DNA, 351 bp, Artificial Sequence
  Synthetic
caggtgcagctggtgcagagcggcgcggaagtgaaaaaaccgggcgcgagcgtgaaagtgagctgcaaagcgagcggctatacctttaccaactattggattggctgggtgcgccaggcgccgggccagggcctggaatggatgggcgatatttatccgggcggcggctataccaactataacgaaaaatttaaaggccgcgtgaccatgacccgcgataccagcaccagcaccgtgtatatggaactgagcagcctgcgcagcgaagataccgcggtgtattattgcgcgcgcggctatgattttgtgctggatcgctggggccagggcaccctggtgaccgtgagcagc

SEQ ID NO: 201 - DNA, 351 bp, Artificial Sequence
  Synthetic
caggtgcagctggtgcagagcggcgcggaagtgaaaaaaccgggcgcgagcgtgaaagtgagctgcaaagcggcgggctatacctttaccaactattggattggctgggtgcgccaggcgccgggccagggcctggaatggatgggcgatatttatccgggcggcggctataccaactataacgaaaaatttaaaggccgcgtgaccatgaccgcggataccagcaccagcaccgtgtatatggaactgagcagcctgcgcagcgaagataccgcggtgtattattgcgcgcgcggctatgattttgtgctggatcgctggggccagggcaccctggtgaccgtgagcagc

SEQ ID NO: 202 - DNA, 351 bp, Artificial Sequence
  Synthetic
caggtgcagctggtgcagagcggcgcggaagtgaaaaaaccgggcgcgagcgtgaaagtgagctgcaaagcgagcggctatacctttaccaactattggattggctgggtgcgccaggcgccgggccagggcctggaatggattggcgatatttatccgggcggcggctataccaactataacgaaaaatttaaaggccgcgtgaccatgaccgcggataccagcaccagcaccgtgtatatggaactgagcagcctgcgcagcgaagataccgcggtgtattattgcgcgcgcggctatgattttgtgctggatcgctggggccagggcaccctggtgaccgtgagcagc

SEQ ID NO: 203 - DNA, 351 bp, Artificial Sequence
  Synthetic
caggtgcagctggtgcagagcggcgcggaagtgaaaaaaccgggcgcgagcgtgaaagtgagctgcaaagcgagcggctatacctttaccaactattggattggctggattcgccaggcgccgggccagggcctggaatggattggcgatatttatccgggcggcggctataccaactataacgaaaaatttaaaggccgcgcgaccctgaccgcggataccagcaccagcaccgtgtatatggaagtgagcagcctgcgcagcgaagataccgcggtgtattattgcgcgcgcggctatgattttgtgctggatcgctggggccagggcaccctggtgaccgtgagcagc

SEQ ID NO: 204 - DNA, 336 bp, Artificial Sequence
  Synthetic
gatgtggtgatgacccagagcccggcgtttctgagcgtgaccccgggcgaaaaagtgaccattacctgcaaaagcagccagagcctgtttaacagcgaaacccagaaaaactatctggcgtggtatcagcagaaaccgggccagccgccgaaactgctgatttattgggcgagcacccgcgaaagcggcgtgccgagccgctttagcggcagcggcagcggcaccgattttaccctgaccattagcagcctgcagccggaagattttgcgacctattattgcaaacagagctataccctgcgcacctttggcggcggcaccaaactggaaattaaa

SEQ ID NO: 205 - DNA, 336 bp, Artificial Sequence; identical to SEQ ID NO: 204
  Synthetic

SEQ ID NO: 206 - DNA, 336 bp, Artificial Sequence
  Synthetic
gatgtggtgatgacccagagcccggcgtttctgagcgtgaccccgggcgaaaaagtgaccattacctgcaaaagcagccagagcctgtttaacagcgaaacccagaaaaactatctggcgtggtatcagcagaaaccgggccagccgccgaaactgctgatttattgggcgagcacccgcgaaagcggcgtgccgagccgctttagcggcagcggcagcggcaccgattttacctttaccattagcagcctggaagcggaagatgcggcgacctattattgcaaacagagctataccctgcgcacctttggcggcggcaccaaactggaaattaaa

SEQ ID NO: 207 - DNA, 336 bp, Artificial Sequence
  Synthetic
gatgtggtgatgacccagagcccggcgtttctgagcgtgaccccgggcgaaaaagtgaccattacctgcaaaagcagccagagcctgtttaacagcgaaacccagaaaaactatctggcgtggtatcagcagaaaccgggccaggcgccgcgcctgctgatttattgggcgagcacccgcgaaagcggcgtgccgagccgctttagcggcagcggcagcggcaccgattttacctttaccattagcagcctggaagcggaagatgcggcgacctattattgcaaacagagctataccctgcgcacctttggcggcggcaccaaactggaaattaaa

SEQ ID NO: 208 - DNA, 336 bp, Artificial Sequence
  Synthetic
gatgtggtgatgacccagagcccggcgtttctgagcgtgaccccgggcgaaaaagtgaccattacctgcaaaagcagccagagcctgtttaacagcgaaacccagaaaaactatctggcgtggtatcagcagaaaccgggccaggcgccgcgcctgctgatttattgggcgagcacccgcgaaagcggcgtgccgagccgctttagcggcagcggcagcggcaccgattttaccctgaccattagcagcctgcagccggaagattttgcgacctattattgcaaacagagctataccctgcgcacctttggcggcggcaccaaactggaaattaaa

SEQ ID NO: 209 - DNA, 336 bp, Artificial Sequence
  Synthetic
gatattcagatgacccagagcccgagcagcctgagcgcgagcgtgggcgatcgcgtgaccattacctgcaaaagcagccagagcctgtttaacagcgaaacccagaaaaactatctggcgtggtatcagcagaaaccgggccagccgccgaaactgctgatttattgggcgagcacccgcgaaagcggcgtgccgagccgctttagcggcagcggcagcggcaccgattttaccctgaccattagcagcctgcagccggaagattttgcgacctattattgcaaacagagctataccctgcgcacctttggcggcggcaccaaactggaaattaaa

SEQ ID NO: 210 - DNA, 336 bp, Artificial Sequence; identical to SEQ ID NO: 204
  Synthetic

SEQ ID NO: 211 - DNA, 336 bp, Artificial Sequence; identical to SEQ ID NO: 206
  Synthetic

SEQ ID NO: 212 - DNA, 336 bp, Artificial Sequence
  Synthetic
gatattgtgatgacccagagcccggatagcctggcggtgagcctgggcgaacgcgcgaccattaactgcaaaagcagccagagcctgtttaacagcgaaacccagaaaaactatctggcgtggtatcagcagaaaccgggccagccgccgaaactgctgatttattgggcgagcacccgcgaaagcggcgtgccggatcgctttagcggcagcggcagcggcaccgattttaccctgaccattagcagcctgcaggcggaagatgtggcggtgtattattgcaaacagagctataccctgcgcacctttggccagggcaccaaactggaaattaaa

SEQ ID NO: 213 - DNA, 336 bp, Artificial Sequence
  Synthetic
gatattgtgatgacccagagcccggatagcctggcggtgagcctgggcgaacgcgcgaccattacctgcaaaagcagccagagcctgtttaacagcgaaacccagaaaaactatctggcgtggtatcagcagaaaccgggccagccgccgaaactgctgattttttgggcgagcacccgcgaaagcggcgtgccggatcgctttctgggcagcggcagcggcaccgattttaccctgaccattagcagcctgcaggcggaagatgtggcggtgtattattgcaaacagagctataccctgcgcacctttggccagggcaccaaactggaaattaaa

SEQ ID NO: 214 - DNA, 336 bp, Artificial Sequence; identical to SEQ ID NO: 212
  Synthetic

SEQ ID NO: 215 - DNA, 336 bp, Artificial Sequence
  Synthetic
gatattgtgatgacccagagcccggatagcctggcggtgagcctgggcgaacgcgcgaccattacctgcaaaagcagccagagcctgtttaacagcgaaacccagaaaaactatctggcgtggtatcagcagaaaccgggccagccgccgaaactgctgattttttgggcgagcacccgcgaaagcggcgtgccggatcgctttagcggcagcggcagcggcaccgattttaccctgaccattagcagcctgcaggcggaagatgtggcggtgtattattgcaaacagagctataccctgcgcacctttggccagggcaccaaactggaaattaaa

SEQ ID NO: 216 - DNA, 336 bp, Artificial Sequence
  Synthetic
gatattgtgatgacccagagcccggatagcctggcggtgagcctgggcgaacgcgcgaccatgacctgcaaaagcagccagagcctgtttaacagcgaaacccagaaaaactatctggcgtggtatcagcagaaaccgggccagccgccgaaactgctgattttttgggcgagcacccgcgaaagcggcgtgccggatcgctttagcggcagcggcagcggcaccgattttaccctgaccattagcagcgtgcaggcggaagatgtggcggtgtattattgcaaacagagctataccctgcgcacctttggccagggcaccaaactggaaattaaa

SEQ ID NO: 217 - DNA, 357 bp, Artificial Sequence
  Synthetic
gtgcatgaagtgcagctggtgcagagcggcgcggaagtgaaaaaaccgggcgaaagcctgaaaattagctgcaaaggcagcggctatagctttaccaacttttatattcattgggtgcgccaggcgccgggccagcgcctggaatggatgggcagcatttatccgaactatggcgataccgcgtataaccagaaatttaaagatcgctttgtgtttagcctggataccagcgtgagcaccgcgtatctgcagattagcagcctgaaagcggaagataccgcggtgtattattgcgcgcgcggctatagctatgcgatggattattggggccagggcaccaccgtgaccgtgagcagc

SEQ ID NO: 218 - DNA, 351 bp, Artificial Sequence
  Synthetic
gaagtgcagctggtgcagagcggcgcggaagtgaaaaaaccgggcgaaagcctgaaaattagctgcaaaggcagcggctatagctttaccaacttttatattcattgggtgcgccaggcgcgcggccagcgcctggaatggattggcagcatttatccgaactatggcgataccgcgtataaccagaaatttaaagatcgctttgtgtttagcctggataccagcgtgagcaccgcgtatctgcagattagcagcctgaaagcggaagataccgcggtgtattattgcgcgcgcggctatagctatgcgatggattattggggccagggcaccaccgtgaccgtgagcagc

SEQ ID NO: 219 - DNA, 351 bp, Artificial Sequence
  Synthetic
gaagtgcagctggtgcagagcggcgcggaagtgaaaaaaccgggcgaaagcctgaaaattagctgcaaaggcagcggctatagctttaccaacttttatattcattgggtgcgccaggcgccgggccagcgcctggaatggatgggcagcatttatccgaactatggcgataccgcgtataaccagaaatttaaagatcgctttgtgtttagcctggataccagcgtgagcaccgcgtatctgcagattagcagcctgaaagcggaagataccgcggtgtattattgcgcgcgcggctatagctatgcgatggattattggggccagggcaccaccgtgaccgtgagcagc

SEQ ID NO: 220 - DNA, 351 bp, Artificial Sequence
  Synthetic
gaagtgcagctggtgcagagcggcgcggaagtgaaaaaaccgggcgcgaccgtgaaaattagctgcaaagtgagcggctatacctttaccaacttttatattcattgggtgcgccaggcgcgcggccagcgcctggaatggattggcagcatttatccgaactatggcgataccgcgtataaccagaaatttaaagatcgcgtgaccattaccgcggataaaagcaccagcaccgcgtatatggaactgagcagcctgcgcagcgaagataccgcggtgtattattgcgcgcgcggctatagctatgcgatggattattggggccagggcaccaccgtgaccgtgagcagc

SEQ ID NO: 221 - DNA, 351 bp, Artificial Sequence
  Synthetic
gaagtgcagctggtgcagagcggcgcggaagtgaaaaaaccgggcgcgaccgtgaaaattagctgcaaagtgagcggctatacctttaccaacttttatattcattgggtgcgccaggcgccgggcaaaggcctggaatggatgggcagcatttatccgaactatggcgataccgcgtataaccagaaatttaaagatcgcgtgaccattaccgcggataaaagcaccagcaccgcgtatatggaactgagcagcctgcgcagcgaagataccgcggtgtattattgcgcgcgcggctatagctatgcgatggattattggggccagggcaccaccgtgaccgtgagcagc

SEQ ID NO: 222 - DNA, 351 bp, Artificial Sequence
  Synthetic
gaagtgcagctggtgcagagcggcgcggaagtgaaaaaaccgggcgaaagcctgaaaattagctgcaaaggcagcggctatagctttaccaacttttatattcattgggtgcgccagatgccgggcaaaggcctggaatggatgggcagcatttatccgaactatggcgataccgcgtataaccagaaatttaaagatcgcgtgaccattaccgcggataaaagcaccagcaccgcgtatatggaactgagcagcctgcgcagcgaagataccgcggtgtattattgcgcgcgcggctatagctatgcgatggattattggggccagggcaccaccgtgaccgtgagcagc

SEQ ID NO: 223 - DNA, 351 bp, Artificial Sequence
  Synthetic
gaagtgcagctggtgcagagcggcgcggaagtgaaaaaaccgggcgaaagcctgaaaattagctgcaaaggcagcggctatagctttaccaacttttatattcattgggtgcgccagatgccgggcaaaggcctggaatggatgggcagcatttatccgaactatggcgataccgcgtataaccagaaatttaaagatcgctttgtgtttagcctggataccagcgtgagcaccgcgtatctgcagattagcagcctgaaagcggaagataccgcggtgtattattgcgcgcgcggctatagctatgcgatggattattggggccagggcaccaccgtgaccgtgagcagc

SEQ ID NO: 224 - DNA, 351 bp, Artificial Sequence; identical to SEQ ID NO: 223
  Synthetic

SEQ ID NO: 225 - DNA, 351 bp, Artificial Sequence
  Synthetic
caggtgcagctggtgcagagcggcgcggaagtgaaaaaaccgggcgcgagcgtgaaagtgagctgcaaagcgagcggctatacctttaccaacttttatattcattgggtgcgccaggcgccgggccagggcctggaatggatgggcagcatttatccgaactatggcgataccgcgtataaccagaaatttaaagatcgcgtgaccatgacccgcgataccagcaccagcaccgtgtatatggaactgagcagcctgcgcagcgaagataccgcggtgtattattgcgcgcgcggctatagctatgcgatggattattggggccagggcaccctggtgaccgtgagcagc

SEQ ID NO: 226 - DNA, 351 bp, Artificial Sequence
  Synthetic
caggtgcagctggtgcagagcggcgcggaagtgaaaaaaccgggcgcgagcgtgaaagtgagctgcaaagcgagcggctatacctttaccaacttttatattcattgggtgcgccaggcgccgggccagggcctggaatggatgggcagcatttatccgaactatggcgataccgcgtataaccagaaatttaaagatcgcgtgaccatgaccgtggataaaagcaccagcaccgtgtatatggaactgcgcagcctgcgcagcgaagataccgcggtgtattattgcgcgcgcggctatagctatgcgatggattattggggccagggcaccctggtgaccgtgagcagc

SEQ ID NO: 227 - DNA, 351 bp, Artificial Sequence
  Synthetic
caggtgcagctggtgcagagcggcgcggaagtgaaaaaaccgggcgcgagcgtgaaagtgagctgcaaagcgagcggctatacctttaccaacttttatattcattgggtgaaacaggcgcatggccagggcctggaatggatgggcagcatttatccgaactatggcgataccgcgtataaccagaaatttaaagatcgcgtgaccatgaccgtggataaaagcaccagcaccgtgtatatggaactgcgcagcctgcgcagcgaagataccgcggtgtattattgcgcgcgcggctatagctatgcgatggattattggggccagggcaccctggtgaccgtgagcagc

SEQ ID NO: 228 - DNA, 351 bp, Artificial Sequence
  Synthetic
caggtgcagctggtgcagagcggcgcggaagtgaaaaaaccgggcgcgagcgtgaaagtgagctgcaaagcgagcggctatacctttaccaacttttatattcattgggtgcgccaggcgccgggccagggcctggaatggattggcagcatttatccgaactatggcgataccgcgtataaccagaaatttaaagatcgcgtgaccatgaccgtggataccagcaccagcaccgtgtatatggaactgagcagcctgcgcagcgaagataccgcggtgtattattgcgcgcgcggctatagctatgcgatggattattggggccagggcaccctggtgaccgtgagcagc

SEQ ID NO: 229 - DNA, 351 bp, Artificial Sequence
  Synthetic
caggtgcagctggtgcagagcggcgcggaagtgaaaaaaccgggcgcgagcgtgaaaatgagctgcaaagcgagcggctatacctttaccaacttttatattcattgggtgcgccaggcgccgggccagggcctggaatggattggcagcatttatccgaactatggcgataccgcgtataaccagaaatttaaagatcgcgcgaccctgaccgtggataccagcaccagcaccgcgtatatggaactgagcagcctgcgcagcgaagataccgcggtgtattattgcgcgcgcggctatagctatgcgatggattattggggccagggcaccctggtgaccgtgagcagc

SEQ ID NO: 230 - DNA, 351 bp, Artificial Sequence
  Synthetic
caggtgcagctggtgcagagcggcgcggaagtgaaaaaaccgggcgcgagcgtgaaaatgagctgcaaagcgagcggctatacctttaccaacttttatattcattgggtgcgccaggcgccgggccagggcctggaatggattggcagcatttatccgaactatggcgataccgcgtataaccagaaatttaaagatcgcgcgaccctgaccgtggataaaagcaccagcaccgcgtatatggaactgagcagcctgcgcagcgaagataccgcggtgtattattgcgcgcgcggctatagctatgcgatggattattggggccagggcaccctggtgaccgtgagcagc

SEQ ID NO: 231 - DNA, 321 bp, Artificial Sequence
  Synthetic
gatattcagatgacccagagcccgagcagcgtgagcgcgagcgtgggcgatcgcgtgaccattacctgcagcgcgagccagggcattagcggcgatctgaactggtatcagcagaaaccgggccaggcgccgcgcctgctgatttatcataccagcagcctgcatagcggcgtgccgagccgctttagcggcagcggcagcggcaccgattttaccctgaccattagcagcctgcagccggaagattttgcgacctattattgccagtattatagcaaagatctgctgacctttggcggcggcaccaaactggaaattaaa

SEQ ID NO: 232 - DNA, 321 bp, Artificial Sequence
  Synthetic
gatattcagatgacccagagcccgagcagcctgagcgcgagcgtgggcgatcgcgtgaccattacctgcagcgcgagccagggcattagcggcgatctgaactggtatcagcagaaaccgggcaaaaccccgaaactgctgatttatcataccagcagcctgcatagcggcgtgccgagccgctttagcggcagcggcagcggcaccgattttaccctgaccattagcagcctgcagccggaagattttgcgacctattattgccagtattatagcaaagatctgctgacctttggcggcggcaccaaactggaaattaaa

SEQ ID NO: 233 - DNA, 321 bp, Artificial Sequence
  Synthetic
gatattcagatgacccagagcccgagcagcgtgagcgcgagcgtgggcgatcgcgtgaccattacctgcagcgcgagccagggcattagcggcgatctgaactggtatcagcagaaaccgggcaaagcgccgaaactgctgatttatcataccagcagcctgcatagcggcgtgccgagccgctttagcggcagcggcagcggcaccgattttaccctgaccattagcagcctgcagccggaagattttgcgacctattattgccagtattatagcaaagatctgctgacctttggcggcggcaccaaactggaaattaaa

SEQ ID NO: 234 - DNA, 321 bp, Artificial Sequence
  Synthetic
gatattcagatgacccagagcccgagcagcgtgagcgcgagcgtgggcgatcgcgtgaccattacctgcagcgcgagccagggcattagcggcgatctgaactggtatcagcagaaaccgggccaggcgccgcgcctgctgatttatcataccagcagcctgcatagcggcgtgccgagccgctttagcggcagcggcagcggcaccgaatttaccctgaccattagccgcctggaaccggaagattttgcggtgtattattgccagtattatagcaaagatctgctgacctttggcggcggcaccaaactggaaattaaa

SEQ ID NO: 235 - DNA, 321 bp, Artificial Sequence
  Synthetic
gatattcagatgacccagagcccgagcaccctgagcgcgagcgtgggcgatcgcgtgaccattacctgcagcgcgagccagggcattagcggcgatctgaactggtatcagcagaaaccgggccaggcgccgcgcctgctgatttatcataccagcagcctgcatagcggcgtgccgagccgctttagcggcagcggcagcggcaccgattttaccctgaccattagcagcctgcagccggaagattttgcgacctattattgccagtattatagcaaagatctgctgacctttggcggcggcaccaaactggaaattaaa

SEQ ID NO: 236 - DNA, 321 bp, Artificial Sequence
  Synthetic
gatattcagatgacccagagcccgagcagcgtgagcgcgagcgtgggcgatcgcgtgaccattacctgcagcgcgagccagggcattagcggcgatctgaactggtatcagcagaaaccgggccaggcgccgcgcctgctgatttatcataccagcagcctgcatagcggcattccggcgcgctttagcggcagcggcagcggcaccgattttaccctgaccattagccgcctggaaccggaagattttgcggtgtattattgccagtattatagcaaagatctgctgacctttggcggcggcaccaaactggaaattaaa

SEQ ID NO: 237 - DNA, 321 bp, Artificial Sequence
  Synthetic
gatattcagatgacccagagcccgagcaccctgagcgcgagcgtgggcgatcgcgtgaccattacctgcagcgcgagccagggcattagcggcgatctgaactggtatcagcagaaaccgggcaaaaccccgaaactgctgatttatcataccagcagcctgcatagcggcgtgccgagccgctttagcggcagcggcagcggcaccgattttaccctgaccattagcagcctgcagccggaagattttgcgacctattattgccagtattatagcaaagatctgctgacctttggcggcggcaccaaactggaaattaaa

SEQ ID NO: 238 - DNA, 321 bp, Artificial Sequence
  Synthetic
gatattcagatgacccagagcccgagcaccctgagcgcgagcgtgggcgatcgcgtgaccattacctgcagcgcgagccagggcattagcggcgatctgaactggtatcagcagaaaccgggccaggcgccgcgcctgctgatttatcataccagcagcctgcatagcggcattccggcgcgctttagcggcagcggcagcggcaccgattttaccctgaccattagcagcctgcagccggaagattttgcggtgtattattgccagtattatagcaaagatctgctgacctttggcggcggcaccaaactggaaattaaa

SEQ ID NO: 239 - DNA, 321 bp, Artificial Sequence
  Synthetic
gatattcagatgacccagagcccgagcagcctgagcgcgagcgtgggcgatcgcgtgaccattacctgcagcgcgagccagggcattagcggcgatctgaactggtatcagcagaaaccgggcaaagcgccgaaactgctgatttatcataccagcagcctgcatagcggcgtgccgagccgctttagcggcagcggcagcggcaccgattttaccctgaccattagcagcctgcagccggaagattttgcgacctattattgccagtattatagcaaagatctgctgacctttggcggcggcaccaaactggaaattaaa

SEQ ID NO: 240 - DNA, 321 bp, Artificial Sequence
  Synthetic
gatattcagatgacccagagcccgagcagcctgagcgcgagcgtgggcgatcgcgtgaccattacctgcagcgcgagccagggcattagcggcgatctgaactggtatcagcagaaaccgggcaaagcggtgaaactgctgatttatcataccagcagcctgcatagcggcgtgccgctgcgctttagcggcagcggcagcggcaccgattataccctgaccattagcagcctgcagccggaagattttgcgacctattattgccagtattatagcaaagatctgctgacctttggcggcggcaccaaactggaaattaaa

SEQ ID NO: 241 - DNA, 321 bp, Artificial Sequence
  Synthetic
gatattcagatgacccagagcccgagcagcctgagcgcgagcgtgggcgatcgcgtgaccattacctgcagcgcgagccagggcattagcggcgatctgaactggtatcagcagaaaagcgatggcgcggtgaaactgctgatttatcataccagcagcctgcatagcggcgtgccgctgcgctttagcggcagcggcagcggcaccgattataccctgaccattagcagcctgcagccggaagattttgcgacctattattgccagtattatagcaaagatctgctgacctttggcggcggcaccaaactggaaattaaa

SEQ ID NO: 242 - DNA, 321 bp, Artificial Sequence
  Synthetic
gatattcagatgacccagagcccgagcagcctgagcgcgagcgtgggcgatcgcgtgaccattacctgcagcgcgagccagggcattagcggcgatctgaactggtatcagcagaaaccgggcaaagcgccgaaactgctgatttatcataccagcagcctgcatagcggcgtgccgagccgctttagcggcagcggcagcggcaccgattataccctgaccattagcagcctgcagccggaagattttgcgacctattattgccagtattatagcaaagatctgctgacctttggcggcggcaccaaactggaaattaaa

SEQ ID NO: 243 - DNA, 360 bp, Artificial Sequence
  Synthetic
gatattcagatgacccagagcccgagcagcctgagcgcgagcgtgggcgatcgcgtgaccattacctgcagcgcgagccagggcattagcggcgatctgaactggtatcagcagaaaccgggcaaagcggtgaaactgctgatttatcataccagcagcctgcatagcggcgtgccgagccgctttagcggcagcggcagcggcaccgattataccctgaccattagcagcctgcagccggaagattttgcgacctattattgccagtattatagcaaagatctgctgacctttggcggcggcaccaaactggaactgaaaaaactgatgaacccgcagcgcagcaccgtgtggtattaa

SEQ ID NO: 244 - protein, 288 aa, Homo sapiens
MQIPQAPWPVVWAVLQLGWRPGWFLASPARPWNPPTFSPALLVVTEGDNATFTCSFSNTSESFVLNWYRMSPSNQTDKLAAFPEDRSQPGQDCRFRVTQLPNGRDFHMSVVRARRNDSGTYLCGAISLAPKAQIKESLRAELRVTERRAEVPTAHPSPSPRPAGQFQTLVVGVVGGLLGSLVLLVWVLAVICSRAARGTIGARRTGQPLKEDPSAVPVFSVDYGELDFQWREKTPEPPVPCVPEQTEYATIVFPSGMGTSSPARRGSADGPRSAQPLRPEDGHCSWPL

SEQ ID NO: 245 - protein, 288 aa, Homo sapiens
MQIPQAPWPVVWAVLQLGWRPGWFLDSPDAPANPPTFSPALLVVTEGDNATFTCSFSNTSESFVLNWYRMSPSNQTDKLAAFPEDRSQPGQDCRFRVTQLPNGRDFHMSVVRARRNDSGTYLCGAISLAPKAQIKESLRAELRVTERRAEVPTAHPSPSPRPAGQFQTLVVGVVGGLLGSLVLLVWVLAVICSRAARGTIGARRTGQPLKEDPSAVPVFSVDYGELDFQWREKTPEPPVPCVPEQTEYATIVFPSGMGTSSPARRGSADGPRSAQPLRPEDGHCSWPL

SEQ ID NO: 246 - protein, 288 aa, Homo sapiens
MQIPQAPWPVVWAVLQLGWRPGWFLDSPDRPWNPPKFSPALLVVTEGDNATFTCSFSNTSESFVLNWYRMSPSNQTDKLAAFPEDRSQPGQDCRFRVTQLPNGRDFHMSVVRARRNDSGTYLCGAISLAPKAQIKESLRAELRVTERRAEVPTAHPSPSPRPAGQFQTLVVGVVGGLLGSLVLLVWVLAVICSRAARGTIGARRTGQPLKEDPSAVPVFSVDYGELDFQWREKTPEPPVPCVPEQTEYATIVFPSGMGTSSPARRGSADGPRSAQPLRPEDGHCSWPL

SEQ ID NO: 247 - protein, 288 aa, Homo sapiens
MQIPQAPWPVVWAVLQLGWRPGWFLDSPDRPWNPPTFAAAALVVTEGDNATFTCSFSNTSESFVLNWYRMSPSNQTDKLAAFPEDRSQPGQDCRFRVTQLPNGRDFHMSVVRARRNDSGTYLCGAISLAPKAQIKESLRAELRVTERRAEVPTAHPSPSPRPAGQFQTLVVGVVGGLLGSLVLLVWVLAVICSRAARGTIGARRTGQPLKEDPSAVPVFSVDYGELDFQWREKTPEPPVPCVPEQTEYATIVFPSGMGTSSPARRGSADGPRSAQPLRPEDGHCSWPL

SEQ ID NO: 248 - protein, 288 aa, Homo sapiens
MQIPQAPWPVVWAVLQLGWRPGWFLDSPDRPWNPPTFSPALLVVTEGANATFTCSFSNTSESFVLNWYRMSPSNQTDKLAAFPEDRSQPGQDCRFRVTQLPNGRDFHMSVVRARRNDSGTYLCGAISLAPKAQIKESLRAELRVTERRAEVPTAHPSPSPRPAGQFQTLVVGVVGGLLGSLVLLVWVLAVICSRAARGTIGARRTGQPLKEDPSAVPVFSVDYGELDFQWREKTPEPPVPCVPEQTEYATIVFPSGMGTSSPARRGSADGPRSAQPLRPEDGHCSWPL

SEQ ID NO: 249 - protein, 288 aa, Homo sapiens
MQIPQAPWPVVWAVLQLGWRPGWFLDSPDRPWNPPTFSPALLVVTEGDAAAFTCSFSNTSESFVLNWYRMSPSNQTDKLAAFPEDRSQPGQDCRFRVTQLPNGRDFHMSVVRARRNDSGTYLCGAISLAPKAQIKESLRAELRVTERRAEVPTAHPSPSPRPAGQFQTLVVGVVGGLLGSLVLLVWVLAVICSRAARGTIGARRTGQPLKEDPSAVPVFSVDYGELDFQWREKTPEPPVPCVPEQTEYATIVFPSGMGTSSPARRGSADGPRSAQPLRPEDGHCSWPL

SEQ ID NO: 250 - protein, 288 aa, Homo sapiens
MQIPQAPWPVVWAVLQLGWRPGWFLDSPDRPWNPPTFSPALLVVTEGDNATAACAFSNTSESFVLNWYRMSPSNQTDKLAAFPEDRSQPGQDCRFRVTQLPNGRDFHMSVVRARRNDSGTYLCGAISLAPKAQIKESLRAELRVTERRAEVPTAHPSPSPRPAGQFQTLVVGVVGGLLGSLVLLVWVLAVICSRAARGTIGARRTGQPLKEDPSAVPVFSVDYGELDFQWREKTPEPPVPCVPEQTEYATIVFPSGMGTSSPARRGSADGPRSAQPLRPEDGHCSWPL

SEQ ID NO: 251 - protein, 288 aa, Homo sapiens
MQIPQAPWPVVWAVLQLGWRPGWFLDSPDRPWNPPTFSPALLVVTEGDNATFTCSFAATSESFVLNWYRMSPSNQTDKLAAFPEDRSQPGQDCRFRVTQLPNGRDFHMSVVRARRNDSGTYLCGAISLAPKAQIKESLRAELRVTERRAEVPTAHPSPSPRPAGQFQTLVVGVVGGLLGSLVLLVWVLAVICSRAARGTIGARRTGQPLKEDPSAVPVFSVDYGELDFQWREKTPEPPVPCVPEQTEYATIVFPSGMGTSSPARRGSADGPRSAQPLRPEDGHCSWPL

SEQ ID NO: 252 - protein, 288 aa, Homo sapiens
MQIPQAPWPVVWAVLQLGWRPGWFLDSPDRPWNPPTFSPALLVVTEGDNATFTCSFSNTSAAFVLNWYRMSPSNQTDKLAAFPEDRSQPGQDCRFRVTQLPNGRDFHMSVVRARRNDSGTYLCGAISLAPKAQIKESLRAELRVTERRAEVPTAHPSPSPRPAGQFQTLVVGVVGGLLGSLVLLVWVLAVICSRAARGTIGARRTGQPLKEDPSAVPVFSVDYGELDFQWREKTPEPPVPCVPEQTEYATIVFPSGMGTSSPARRGSADGPRSAQPLRPEDGHCSWPL

SEQ ID NO: 253 - protein, 288 aa, Homo sapiens
MQIPQAPWPVVWAVLQLGWRPGWFLDSPDRPWNPPTFSPALLVVTEGDNATFTCSFSNTSESFALAWARMSPSNQTDKLAAFPEDRSQPGQDCRFRVTQLPNGRDFHMSVVRARRNDSGTYLCGAISLAPKAQIKESLRAELRVTERRAEVPTAHPSPSPRPAGQFQTLVVGVVGGLLGSLVLLVWVLAVICSRAARGTIGARRTGQPLKEDPSAVPVFSVDYGELDFQWREKTPEPPVPCVPEQTEYATIVFPSGMGTSSPARRGSADGPRSAQPLRPEDGHCSWPL

SEQ ID NO: 254 - protein, 288 aa, Homo sapiens
MQIPQAPWPVVWAVLQLGWRPGWFLDSPDRPWNPPTFSPALLVVTEGDNATFTCSFSNTSESFVLNWYRMSPANAADKLAAFPEDRSQPGQDCRFRVTQLPNGRDFHMSVVRARRNDSGTYLCGAISLAPKAQIKESLRAELRVTERRAEVPTAHPSPSPRPAGQFQTLVVGVVGGLLGSLVLLVWVLAVICSRAARGTIGARRTGQPLKEDPSAVPVFSVDYGELDFQWREKTPEPPVPCVPEQTEYATIVFPSGMGTSSPARRGSADGPRSAQPLRPEDGHCSWPL

SEQ ID NO: 255 - protein, 288 aa, Homo sapiens
MQIPQAPWPVVWAVLQLGWRPGWFLDSPDRPWNPPTFSPALLVVTEGDNATFTCSFSNTSESFVLNWYRMSPSNQADALAAFPEDRSQPGQDCRFRVTQLPNGRDFHMSVVRARRNDSGTYLCGAISLAPKAQIKESLRAELRVTERRAEVPTAHPSPSPRPAGQFQTLVVGVVGGLLGSLVLLVWVLAVICSRAARGTIGARRTGQPLKEDPSAVPVFSVDYGELDFQWREKTPEPPVPCVPEQTEYATIVFPSGMGTSSPARRGSADGPRSAQPLRPEDGHCSWPL

SEQ ID NO: 256 - protein, 288 aa, Homo sapiens
MQIPQAPWPVVWAVLQLGWRPGWFLDSPDRPWNPPTFSPALLVVTEGDNATFTCSFSNTSESFVLNWYRMSPSNQTDKLAAFPEAASQPGQDCRFRVTQLPNGRDFHMSVVRARRNDSGTYLCGAISLAPKAQIKESLRAELRVTERRAEVPTAHPSPSPRPAGQFQTLVVGVVGGLLGSLVLLVWVLAVICSRAARGTIGARRTGQPLKEDPSAVPVFSVDYGELDFQWREKTPEPPVPCVPEQTEYATIVFPSGMGTSSPARRGSADGPRSAQPLRPEDGHCSWPL

SEQ ID NO: 257 - protein, 288 aa, Homo sapiens
MQIPQAPWPVVWAVLQLGWRPGWFLDSPDRPWNPPTFSPALLVVTEGDNATFTCSFSNTSESFVLNWYRMSPSNQTDKLAAFPEDRSQAAGDCRFRVTQLPNGRDFHMSVVRARRNDSGTYLCGAISLAPKAQIKESLRAELRVTERRAEVPTAHPSPSPRPAGQFQTLVVGVVGGLLGSLVLLVWVLAVICSRAARGTIGARRTGQPLKEDPSAVPVFSVDYGELDFQWREKTPEPPVPCVPEQTEYATIVFPSGMGTSSPARRGSADGPRSAQPLRPEDGHCSWPL

SEQ ID NO: 258 - protein, 288 aa, Homo sapiens
MQIPQAPWPVVWAVLQLGWRPGWFLDSPDRPWNPPTFSPALLVVTEGDNATFTCSFSNTSESFVLNWYRMSPSNQTDKLAAFPEDRSQPGAACRFRVTQLPNGRDFHMSVVRARRNDSGTYLCGAISLAPKAQIKESLRAELRVTERRAEVPTAHPSPSPRPAGQFQTLVVGVVGGLLGSLVLLVWVLAVICSRAARGTIGARRTGQPLKEDPSAVPVFSVDYGELDFQWREKTPEPPVPCVPEQTEYATIVFPSGMGTSSPARRGSADGPRSAQPLRPEDGHCSWPL

SEQ ID NO: 259 - protein, 288 aa, Homo sapiens
MQIPQAPWPVVWAVLQLGWRPGWFLDSPDRPWNPPTFSPALLVVTEGDNATFTCSFSNTSESFVLNWYRMSPSNQTDKLAAFPEDRSQPGQDCRFAVAQLPNGRDFHMSVVRARRNDSGTYLCGAISLAPKAQIKESLRAELRVTERRAEVPTAHPSPSPRPAGQFQTLVVGVVGGLLGSLVLLVWVLAVICSRAARGTIGARRTGQPLKEDPSAVPVFSVDYGELDFQWREKTPEPPVPCVPEQTEYATIVFPSGMGTSSPARRGSADGPRSAQPLRPEDGHCSWPL

SEQ ID NO: 260 - protein, 288 aa, Homo sapiens
MQIPQAPWPVVWAVLQLGWRPGWFLDSPDRPWNPPTFSPALLVVTEGDNATFTCSFSNTSESFVLNWYRMSPSNQTDKLAAFPEDRSQPGQDCRFRVTQLPAGADFHMSVVRARRNDSGTYLCGAISLAPKAQIKESLRAELRVTERRAEVPTAHPSPSPRPAGQFQTLVVGVVGGLLGSLVLLVWVLAVICSRAARGTIGARRTGQPLKEDPSAVPVFSVDYGELDFQWREKTPEPPVPCVPEQTEYATIVFPSGMGTSSPARRGSADGPRSAQPLRPEDGHCSWPL

SEQ ID NO: 261 - protein, 288 aa, Homo sapiens
MQIPQAPWPVVWAVLQLGWRPGWFLDSPDRPWNPPTFSPALLVVTEGDNATFTCSFSNTSESFVLNWYRMSPSNQTDKLAAFPEDRSQPGQDCRFRVTQLPNGRAFHMSVVRARRNDSGTYLCGAISLAPKAQIKESLRAELRVTERRAEVPTAHPSPSPRPAGQFQTLVVGVVGGLLGSLVLLVWVLAVICSRAARGTIGARRTGQPLKEDPSAVPVFSVDYGELDFQWREKTPEPPVPCVPEQTEYATIVFPSGMGTSSPARRGSADGPRSAQPLRPEDGHCSWPL

SEQ ID NO: 262 - protein, 288 aa, Homo sapiens
MQIPQAPWPVVWAVLQLGWRPGWFLDSPDRPWNPPTFSPALLVVTEGDNATFTCSFSNTSESFVLNWYRMSPSNQTDKLAAFPEDRSQPGQDCRFRVTQLPNGRDFAMAVVRARRNDSGTYLCGAISLAPKAQIKESLRAELRVTERRAEVPTAHPSPSPRPAGQFQTLVVGVVGGLLGSLVLLVWVLAVICSRAARGTIGARRTGQPLKEDPSAVPVFSVDYGELDFQWREKTPEPPVPCVPEQTEYATIVFPSGMGTSSPARRGSADGPRSAQPLRPEDGHCSWPL

SEQ ID NO: 263 - protein, 288 aa, Homo sapiens
MQIPQAPWPVVWAVLQLGWRPGWFLDSPDRPWNPPTFSPALLVVTEGDNATFTCSFSNTSESFVLNWYRMSPSNQTDKLAAFPEDRSQPGQDCRFRVTQLPNGRDFHMSVAAARRNDSGTYLCGAISLAPKAQIKESLRAELRVTERRAEVPTAHPSPSPRPAGQFQTLVVGVVGGLLGSLVLLVWVLAVICSRAARGTIGARRTGQPLKEDPSAVPVFSVDYGELDFQWREKTPEPPVPCVPEQTEYATIVFPSGMGTSSPARRGSADGPRSAQPLRPEDGHCSWPL

SEQ ID NO: 264 - protein, 288 aa, Homo sapiens
MQIPQAPWPVVWAVLQLGWRPGWFLDSPDRPWNPPTFSPALLVVTEGDNATFTCSFSNTSESFVLNWYRMSPSNQTDKLAAFPEDRSQPGQDCRFRVTQLPNGRDFHMSVVRAAANDSGTYLCGAISLAPKAQIKESLRAELRVTERRAEVPTAHPSPSPRPAGQFQTLVVGVVGGLLGSLVLLVWVLAVICSRAARGTIGARRTGQPLKEDPSAVPVFSVDYGELDFQWREKTPEPPVPCVPEQTEYATIVFPSGMGTSSPARRGSADGPRSAQPLRPEDGHCSWPL

SEQ ID NO: 265 - protein, 288 aa, Homo sapiens
MQIPQAPWPVVWAVLQLGWRPGWFLDSPDRPWNPPTFSPALLVVTEGDNATFTCSFSNTSESFVLNWYRMSPSNQTDKLAAFPEDRSQPGQDCRFRVTQLPNGRDFHMSVVRARRNASGTYLCGAISLAPKAQIKESLRAELRVTERRAEVPTAHPSPSPRPAGQFQTLVVGVVGGLLGSLVLLVWVLAVICSRAARGTIGARRTGQPLKEDPSAVPVFSVDYGELDFQWREKTPEPPVPCVPEQTEYATIVFPSGMGTSSPARRGSADGPRSAQPLRPEDGHCSWPL

SEQ ID NO: 266 - protein, 288 aa, Homo sapiens
MQIPQAPWPVVWAVLQLGWRPGWFLDSPDRPWNPPTFSPALLVVTEGDNATFTCSFSNTSESFVLNWYRMSPSNQTDKLAAFPEDRSQPGQDCRFRVTQLPNGRDFHMSVVRARRNDSGTYLCAGASAAPKAQIKESLRAELRVTERRAEVPTAHPSPSPRPAGQFQTLVVGVVGGLLGSLVLLVWVLAVICSRAARGTIGARRTGQPLKEDPSAVPVFSVDYGELDFQWREKTPEPPVPCVPEQTEYATIVFPSGMGTSSPARRGSADGPRSAQPLRPEDGHCSWPL

SEQ ID NO: 267 - protein, 288 aa, Homo sapiens
MQIPQAPWPVVWAVLQLGWRPGWFLDSPDRPWNPPTFSPALLVVTEGDNATFTCSFSNTSESFVLNWYRMSPSNQTDKLAAFPEDRSQPGQDCRFRVTQLPNGRDFHMSVVRARRNDSGTYLCGAISLAPTAQIKESLRAELRVTERRAEVPTAHPSPSPRPAGQFQTLVVGVVGGLLGSLVLLVWVLAVICSRAARGTIGARRTGQPLKEDPSAVPVFSVDYGELDFQWREKTPEPPVPCVPEQTEYATIVFPSGMGTSSPARRGSADGPRSAQPLRPEDGHCSWPL

SEQ ID NO: 268 - protein, 288 aa, Homo sapiens
MQIPQAPWPVVWAVLQLGWRPGWFLDSPDRPWNPPTFSPALLVVTEGDNATFTCSFSNTSESFVLNWYRMSPSNQTDKLAAFPEDRSQPGQDCRFRVTQLPNGRDFHMSVVRARRNDSGTYLCGAISLAPKAQITASLRAELRVTERRAEVPTAHPSPSPRPAGQFQTLVVGVVGGLLGSLVLLVWVLAVICSRAARGTIGARRTGQPLKEDPSAVPVFSVDYGELDFQWREKTPEPPVPCVPEQTEYATIVFPSGMGTSSPARRGSADGPRSAQPLRPEDGHCSWPL

SEQ ID NO: 269 - protein, 288 aa, Homo sapiens
MQIPQAPWPVVWAVLQLGWRPGWFLDSPDRPWNPPTFSPALLVVTEGDNATFTCSFSNTSESFVLNWYRMSPSNQTDKLAAFPEDRSQPGQDCRFRVTQLPNGRDFHMSVVRARRNDSGTYLCGAISLAPKAQIKESLAAALRVTERRAEVPTAHPSPSPRPAGQFQTLVVGVVGGLLGSLVLLVWVLAVICSRAARGTIGARRTGQPLKEDPSAVPVFSVDYGELDFQWREKTPEPPVPCVPEQTEYATIVFPSGMGTSSPARRGSADGPRSAQPLRPEDGHCSWPL

SEQ ID NO: 270 - protein, 288 aa, Homo sapiens
MQIPQAPWPVVWAVLQLGWRPGWFLDSPDRPWNPPTFSPALLVVTEGDNATFTCSFSNTSESFVLNWYRMSPSNQTDKLAAFPEDRSQPGQDCRFRVTQLPNGRDFHMSVVRARRNDSGTYLCGAISLAPKAQIKESLRAELRVTARRAEVPTAHPSPSPRPAGQFQTLVVGVVGGLLGSLVLLVWVLAVICSRAARGTIGARRTGQPLKEDPSAVPVFSVDYGELDFQWREKTPEPPVPCVPEQTEYATIVFPSGMGTSSPARRGSADGPRSAQPLRPEDGHCSWPL

SEQ ID NO: 271 - protein, 288 aa, Homo sapiens
MQIPQAPWPVVWAVLQLGWRPGWFLDSPDRPWNPPTFSPALLVVTEGDNATFTCSFSNTSESFVLNWYRMSPSNQTDKLAAFPEDRSQPGQDCRFRVTQLPNGRDFHMSVVRARRNDSGTYLCGAISLAPKAQIKESLRAELRVTEAAAEVPTAHPSPSPRPAGQFQTLVVGVVGGLLGSLVLLVWVLAVICSRAARGTIGARRTGQPLKEDPSAVPVFSVDYGELDFQWREKTPEPPVPCVPEQTEYATIVFPSGMGTSSPARRGSADGPRSAQPLRPEDGHCSWPL

SEQ ID NO: 272 - protein, 288 aa, Homo sapiens
MQIPQAPWPVVWAVLQLGWRPGWFLDSPDRPWNPPTFSPALLVVTEGDNATFTCSFSNTSESFVLNWYRMSPSNQTDKLAAFPEDRSQPGQDCRFRVTQLPNGRDFHMSVVRARRNDSGTYLCGAISLAPKAQIKESLRAELRVTERRAEVPTAAAAPSPRPAGQFQTLVVGVVGGLLGSLVLLVWVLAVICSRAARGTIGARRTGQPLKEDPSAVPVFSVDYGELDFQWREKTPEPPVPCVPEQTEYATIVFPSGMGTSSPARRGSADGPRSAQPLRPEDGHCSWPL

SEQ ID NO: 273 - protein, 288 aa, Homo sapiens
MQIPQAPWPVVWAVLQLGWRPGWFLDSPDRPWNPPTFSPALLVVTEGDNATFTCSFSNTSESFVLNWYRMSPSNQTDKLAAFPEDRSQPGQDCRFRVTQLPNGRDFHMSVVRARRNDSGTYLCGAISLAPKAQIKESLRAELRVTERRAEVPTAHPSPSPAAAGQFQTLVVGVVGGLLGSLVLLVWVLAVICSRAARGTIGARRTGQPLKEDPSAVPVFSVDYGELDFQWREKTPEPPVPCVPEQTEYATIVFPSGMGTSSPARRGSADGPRSAQPLRPEDGHCSWPL

SEQ ID NO: 274 - protein, 288 aa, Homo sapiens
MQIPQAPWPVVWAVLQLGWRPGWFLDSPDRPWNPPTFSPAALLVTEGDNATFTCSFSNTSESFVLNWYRMSPSNQTDKLAAFPEDRSQPGQDCRFRVTQLPNGRDFHMSVVRARRNDSGTYLCGAISLAPKAQIKESLRAELRVTERRAEVPTAHPSPSPRPAGQFQTLVVGVVGGLLGSLVLLVWVLAVICSRAARGTIGARRTGQPLKEDPSAVPVFSVDYGELDFQWREKTPEPPVPCVPEQTEYATIVFPSGMGTSSPARRGSADGPRSAQPLRPEDGHCSWPL

SEQ ID NO: 275 - protein, 288 aa, Homo sapiens
MQIPQAPWPVVWAVLQLGWRPGWFLDSPDRPWNPPTFSPALLVVTEGDNATFTCSFSNTSESFVLNWYRMSPSNQTDKLAAFPEDRSQPGQDCRFRVTQLPNGRDFHMSVVRARRNDSGTYLCGAISLAPKAQIKESLRAELRVTERRAEVPTAHPSPSPRPAGQFQTLVVGVVGGLLGSLVLLVWVLAVICSRAARGTIGARRTGQPLKEDPSAVPVFSVDYGELDFQWREKTPEPPVPCVPEQTEYATIVFPSGMGTSSPARRGSADGPRSAQPLRPEDGHCSWPL

SEQ ID NO: 276 - protein, 288 aa, Macaca mulatta
MQIPQAPWPVVWAVLQLGWRPGWFLESPDRPWNPPTFSPALLLVTEGDNATFTCSFSNASESFVLNWYRMSPSNQTDKLAAFPEDRSQPGRDCRFRVTQLPNGRDFHMSVVRARRNDSGTYLCGAISLAPKAQIKESLRAELRVTERRAEVPTAHPSPSPRPAGQFQALVVGVVGGLLGSLVLLVWVLAVICSRAAQGTIEARRTGQPLKEDPSAVPVFSVDYGELDFQWREKTPEPPAPCVPEQTEYATIVFPSGLGTSSPARRGSADGPRSPRPLRPEDGHCSWPL

SEQ ID NO: 277 - protein, 117 aa, Unknown
  Mouse VH reference sequence
QVQLQQPGAELVRPGTSVKMSCKAAGYTFTNYWIGWIKQRPGHGLEWIGDIYPGGGYTNYNEKFKGKATLTADTSSSTAYMQVSSLTSEDTGIYYCARGYDFVLDRWGQGTSVTVSS

SEQ ID NO: 278 - protein, 112 aa, Unknown
  Mouse VL reference sequence
DIVMSQSPSSLAVSTGEKVTMTCKSSQSLFNSETQKNYLAWYQQKPGQPPKLLIFWASTRESGVPDRFLGSGSGTDFTLTISSVQAEDLAVYYCKQSYTLRTFGGGTKLEIK

SEQ ID NO: 279 - protein, 117 aa, Unknown
  Mouse VH reference sequence
EVQLHQSGPELLKPGASVRMSCKASGYTFTNFYIHWVKQSHGKSIEWIGSIYPNYGDTAYNQKFKDKATLTVDKSSSTAYMALRSLTSEDSAVYYCARGYSYAMDYWGQGTSVTVSS

SEQ ID NO: 280 - protein, 107 aa, Unknown
  Mouse VL reference sequence
NIVMTQSPKSMSMSVGERVTLTCKASENVVTYVSWYQQKPEQSPKLLIYGASNRYTGVPDRFTGSGSATDFTLTISSVQAEDLADYHCGQGYSYPYTFGGGTKLEIK

SEQ ID NO: 281 - protein, 149 aa, Homo sapiens
PGWFLDSPDRPWNPPTFSPALLVVTEGDNATFTCSFSNTSESFVLNWYRMSPSNQTDKLAAFPEDRSQPGQDCRFRVTQLPNGRDFHMSVVRARRNDSGTYLCGAISLAPKAQIKESLRAELRVTERRAEVPTAHPSPSPRPAGQFQTL

SEQ ID NO: 282 - protein, 149 aa, Unknown
  Monkey
PGWFLESPDRPWNPPTFSPALLLVTEGDNATFTCSFSNASESFVLNWYRMSPSNQTDKLAAFPEDRSQPGRDCRFRVTQLPNGRDFHMSVVRARRNDSGTYLCGAISLAPKAQIKESLRAELRVTERRAEVPTAHPSPSPRPAGQFQAL

SEQ ID NO: 283 - protein, 149 aa, Unknown
  Horse
SVHLLDSPDRPWNRPLFSPARLMVPEGANATFTCSFSNTSEHFVLNWYRMSPSNQTDKLAAFPEDSSQPGRSGRFRVTRLPNGRDFHMSVLAARRNDSGIYLCGAISLPPKTQINESPRAELTVTERIPEPPTEHPSPSPSPAGQLQGL

SEQ ID NO: 284 - protein, 149 aa, Unknown
  Dog
PGWLLDSPDRPWSPLTFSPAQLTVQEGENATFTCSLADIPDSFVLNWYRLSPRNQTDKLAAFQEDRIEPGRDRRFRVTRLPNGRDFHMSIVAARLNDSGIYLCGAIYLPPNTQINESPRAELSVTERTLEPPTQSPSPSPRLSGQLQGL

SEQ ID NO: 285 - protein, 149 aa, Unknown
  Mouse
SGWLLEVPNGPWRSLTFYPAWLTVSEGANATFTCSLSNWSEDLMLNWNRLSPSNQTEKQAAFCNGLSQPVQDARFQIIQLPNRHDFHMNILDTRRNDSGIYLCGAISLHPKAKIEESPGAELVVTERILETSTRYPSPSPKPEGRFQGM

SEQ ID NO: 286 - protein, 149 aa, Unknown
  Rat
SGWLLEVLNKPWRPLTFSPTWLTVSEGANATFTCSFSNWSEDLKLNWYRLSPSNQTEKQAAFCNGYSQPVRDARFQIVQLPNGHDFHMNILDARRNDSGIYLCGAISLPPKAQIKESPGAELVVTERILETPTRYPRPSPKPEGQFQGL

SEQ ID NO: 287 - protein, 15 aa, Artificial Sequence
  Synthetic
RASKGVSTSGYSYLH

SEQ ID NO: 288 - protein, 7 aa, Artificial Sequence
  Synthetic
LASYLES

SEQ ID NO: 289 - protein, 9 aa, Artificial Sequence
  Synthetic
QHSRDLPLT

SEQ ID NO: 290 - protein, 5 aa, Artificial Sequence
  Synthetic
NYYMY

SEQ ID NO: 291 - protein, 17 aa, Artificial Sequence
  Synthetic
GINPSNGGTNFNEKFKN

SEQ ID NO: 292 - protein, 11 aa, Artificial Sequence
  Synthetic
RDYRFDMGFDY